European Patent Application EP 4 566 671 A2, published June 11, 2025. Title: CONSTRUCTION AND APPLICATION OF FUSION PROTEIN VACCINE PLATFORM. Applicant: INSTITUTE OF BIOPHYSICS, CHINESE ACADEMY OF SCIENCES. Application EP, filed July 1, 2021. The sequence listing filed with the application follows.

SEQUENCE LISTING (93 sequences)

SEQ ID NO: 1 - protein, 162 aa, Mus musculus
CDLPHTYNLGNKRALTVLEEMRRLPPLSCLKDRKDFGFPLEKVDNQQIQKAQAILVLRDLTQQILNLFTSKDLSATWNATLLDSFCNDLHQQLNDLKACVMQEPPLTQEDSLLAVRTYFHRITVYLRKKKHSLCAWEVIRAEVWRALSSSTNLLARLSEEKE

SEQ ID NO: 2 - protein, 233 aa, Homo sapiens
EPKSCDKTHTCPPCPAPELLGGPSVFLFPPKPKDQLMISRTPEVTCVVVDVSHEDPEVKFNWYVDGVEVHNAKTKPREEQYNSTYRVVSVLTVLHQDWLNGKEYKCKVSNKALPAPIEKTISKAKGQPREPQVYTLPPSRDELTKNQVSLTCLVKGFYPSDIAVEWESNGQPENNYKTTPPVLDSDGSFLYSKLTVDKSRWQQGNVFSCSVLHEALHNHYTQKSLSLSPGKHV

SEQ ID NO: 3 - protein, 13 aa, Homo sapiens
AKFVAAWTLKAAA

SEQ ID NO: 4 - protein, 15 aa, synthetic construct
  REGION 1..15: note = artificially synthesized sequence
GGGGSGGGGSGGGGS

SEQ ID NO: 5 - protein, 24 aa, Homo sapiens
MARLCAFLMILVMMSYYWSACSLG

SEQ ID NO: 6 - protein, 119 aa, HBV
MGGWSSKPRKGMGTNLSVPNPLGFFPDHQLDPAFGANSNNPDWDFNPIKDHWPAANQVGVGAFGPGLTPPHGGILGWSPQAQGILTTVSTIPPPASTNRQSGRQPTPISPPLRDSHPQA

SEQ ID NO: 7 - protein, 226 aa, HBV
MENTTSGFLGPLLVLQAGFFLLTRILTIPQSLDSWWTSLNFLGGAPTCPGQNSQSPTSNHSPTSCPPICPGYRWMCLRRFIIFLFILLLCLIFLLVLLDYQGMLPVCPLLPGTSTTSTGPCKTCTIPAQGTSMFPSCCCTKPSDGNCTCIPIPSSWAFARFLWEWASVRFSWLSLLVPFVQWFVGLSPTVWLSVIWMMWYWGPSLYNILSPFLPLLPIFFCLWVYI

SEQ ID NO: 8 - protein, 223 aa, SARS-CoV-2
RVQPTESIVRFPNITNLCPFGEVFNATRFASVYAWNRKRISNCVADYSVLYNSASFSTFKCYGVSPTKLNDLCFTNVYADSFVIRGDEVRQIAPGQTGKIADYNYKLPDDFTGCVIAWNSNNLDSKVGGNYNYLYRLFRKSNLKPFERDISTEIYQAGSTPCNGVEGFNCYFPLQSYGFQPTNGVGYQPYRVVVLSFELLHAPATVCGPKKSTNLVKNKCVNF

SEQ ID NO: 9 - protein, 326 aa, Influenza virus
DTICIGYHANNSTDTVDTVLEKNVTVTHSVNLLEDSHNGKLCRLKGIAPLQLGKCNIAGWLLGNPECDPLLPVRSWSYIVETPNSENGICYPGDFIDYEELREQLSSVSSFERFEIFPKESSWPNHNTNGVTAACSHEGKSSFYRNLLWLTEKEGSYPKLKNSYVNKKGKEVLVLWGIHHPPNSKEQQNLYQNENAYVSVVTSNYNRRFTPEIAERPKVRDQAGRMNYYWTLLKPGDTIIFEANGNLIAPMYAFALSRGFGSGIITSNASMHECNTKCQTPLGAINSSLPYQNIHPVTIGECPKYVRSAKLRMVTGLRNNPSIQSR

SEQ ID NO: 10 - protein, 98 aa, HPV
MHGDTPTLHEYMLDLQPETTDLYCYEQLNDSSEEEDEIDGPAGQAEPDRAHYNIVTFCCKCDSTLRLCVQSTHVDIRTLEDLLMGTLGIVCPICSQKP

SEQ ID NO: 11 - protein, 527 aa, Mus musculus
CDLPHTYNLGNKRALTVLEEMRRLPPLSCLKDRKDFGFPLEKVDNQQIQKAQAILVLRDLTQQILNLFTSKDLSATWNATLLDSFCNDLHQQLNDLKACVMQEPPLTQEDSLLAVRTYFHRITVYLRKKKHSLCAWEVIRAEVWRALSSSTNLLARLSEEKESGGGGSGGGGSGGGGSGGGGRTMGQNLSTSNPLGFFPDHQLDPAFRANTANPDWDFNPNKDTWPDANKVGAGAFGLGFTPPHGGLLGWSPQAQGILQTLPANPPPASTNRQTGRQPTPLSPPLRNTHPQAFEEPKSCDKTHTCPPCPAPELLGGPSVFLFPPKPKDQLMISRTPEVTCVVVDVSHEDPEVKFNWYVDGVEVHNAKTKPREEQYNSTYRVVSVLTVLHQDWLNGKEYKCKVSNKALPAPIEKTISKAKGQPREPQVYTLPPSRDELTKNQVSLTCLVKGFYPSDIAVEWESNGQPENNYKTTPPVLDSDGSFLYSKLTVDKSRWQQGNVFSCSVLHEALHNHYTQKSLSLSPGKHV

SEQ ID NO: 12 - protein, 642 aa, Mus musculus
CDLPHTYNLGNKRALTVLEEMRRLPPLSCLKDRKDFGFPLEKVDNQQIQKAQAILVLRDLTQQILNLFTSKDLSATWNATLLDSFCNDLHQQLNDLKACVMQEPPLTQEDSLLAVRTYFHRITVYLRKKKHSLCAWEVIRAEVWRALSSSTNLLARLSEEKESGGGGSGGGGSGGGGSGGGGRTRVQPTESIVRFPNITNLCPFGEVFNATRFASVYAWNRKRISNCVADYSVLYNSASFSTFKCYGVSPTKLNDLCFTNVYADSFVIRGDEVRQIAPGQTGKIADYNYKLPDDFTGCVIAWNSNNLDSKVGGNYNYLYRLFRKSNLKPFERDISTEIYQAGSTPCNGVEGFNCYFPLQSYGFQPTNGVGYQPYRVVVLSFELLHAPATVCGPKKSTNLVKNKCVNFFEEPKSCDKTHTCPPCPAPELLGGPSVFLFPPKPKDQLMISRTPEVTCVVVDVSHEDPEVKFNWYVDGVEVHNAKTKPREEQYNSTYRVVSVLTVLHQDWLNGKEYKCKVSNKALPAPIEKTISKAKGQPREPQVYTLPPSRDELTKNQVSLTCLVKGFYPSDIAVEWESNGQPENNYKTTPPVLDSDGSFLYSKLTVDKSRWQQGNVFSCSVLHEALHNHYTQKSLSLSPGKHV

SEQ ID NO: 13 - protein, 745 aa, Mus musculus
CDLPHTYNLGNKRALTVLEEMRRLPPLSCLKDRKDFGFPLEKVDNQQIQKAQAILVLRDLTQQILNLFTSKDLSATWNATLLDSFCNDLHQQLNDLKACVMQEPPLTQEDSLLAVRTYFHRITVYLRKKKHSLCAWEVIRAEVWRALSSSTNLLARLSEEKESGGGGSGGGGSGGGGSGGGGRTDTICIGYHANNSTDTVDTVLEKNVTVTHSVNLLEDSHNGKLCRLKGIAPLQLGKCNIAGWLLGNPECDPLLPVRSWSYIVETPNSENGICYPGDFIDYEELREQLSSVSSFERFEIFPKESSWPNHNTNGVTAACSHEGKSSFYRNLLWLTEKEGSYPKLKNSYVNKKGKEVLVLWGIHHPPNSKEQQNLYQNENAYVSVVTSNYNRRFTPEIAERPKVRDQAGRMNYYWTLLKPGDTIIFEANGNLIAPMYAFALSRGFGSGIITSNASMHECNTKCQTPLGAINSSLPYQNIHPVTIGECPKYVRSAKLRMVTGLRNNPSIQSRFEEPKSCDKTHTCPPCPAPELLGGPSVFLFPPKPKDQLMISRTPEVTCVVVDVSHEDPEVKFNWYVDGVEVHNAKTKPREEQYNSTYRVVSVLTVLHQDWLNGKEYKCKVSNKALPAPIEKTISKAKGQPREPQVYTLPPSRDELTKNQVSLTCLVKGFYPSDIAVEWESNGQPENNYKTTPPVLDSDGSFLYSKLTVDKSRWQQGNVFSCSVLHEALHNHYTQKSLSLSPGKHV

SEQ ID NO: 14 - protein, 517 aa, Mus musculus
CDLPHTYNLGNKRALTVLEEMRRLPPLSCLKDRKDFGFPLEKVDNQQIQKAQAILVLRDLTQQILNLFTSKDLSATWNATLLDSFCNDLHQQLNDLKACVMQEPPLTQEDSLLAVRTYFHRITVYLRKKKHSLCAWEVIRAEVWRALSSSTNLLARLSEEKESGGGGSGGGGSGGGGSGGGGRTMHGDTPTLHEYMLDLQPETTDLYCYEQLNDSSEEEDEIDGPAGQAEPDRAHYNIVTFCCKCDSTLRLCVQSTHVDIRTLEDLLMGTLGIVCPICSQKPFEEPKSCDKTHTCPPCPAPELLGGPSVFLFPPKPKDQLMISRTPEVTCVVVDVSHEDPEVKFNWYVDGVEVHNAKTKPREEQYNSTYRVVSVLTVLHQDWLNGKEYKCKVSNKALPAPIEKTISKAKGQPREPQVYTLPPSRDELTKNQVSLTCLVKGFYPSDIAVEWESNGQPENNYKTTPPVLDSDGSFLYSKLTVDKSRWQQGNVFSCSVLHEALHNHYTQKSLSLSPGKHV

SEQ ID NO: 15 - protein, 411 aa, Mus musculus
CDLPHTYNLGNKRALTVLEEMRRLPPLSCLKDRKDFGFPLEKVDNQQIQKAQAILVLRDLTQQILNLFTSKDLSATWNATLLDSFCNDLHQQLNDLKACVMQEPPLTQEDSLLAVRTYFHRITVYLRKKKHSLCAWEVIRAEVWRALSSSTNLLARLSEEKESGGGGSGGGGSGGGGSGGGGRTDKTHTCPPCPAPELLGGPSVFLFPPKPKDTLMISRTPEVTCVVVDVSHEDPEVKFNWYVDGVEVHNAKTKPREEQYNSTYRVVSVLTVLHQDWLNGKEYKCKVSNKALPAPIEKTISKAKGQPREPQVCTLPPSRDELTKNQVSLSCAVKGFYPSDIAVEWESNGQPENNYKTTPPVLDSDGSFFLVSKLTVDKSRWQQGNVFSCSVMHEALHNHYTQKSLSLSPGK

SEQ ID NO: 16 - protein, 337 aa, Mus musculus
MGQNLSTSNPLGFFPDHQLDPAFRANTANPDWDFNPNKDTWPDANKVGAGAFGLGFTPPHGGLLGWSPQAQGILQTLPANPPPASTNRQTGRQPTPLSPPLRNTHPQAFEDKTHTCPPCPAPELLGGPSVFLFPPKPKDTLMISRTPEVTCVVVDVSHEDPEVKFNWYVDGVEVHNAKTKPREEQYNSTYRVVSVLTVLHQDWLNGKEYKCKVSNKALPAPIEKTISKAKGQPREPQVYTLPPCRDELTKNQVSLWCLVKGFYPSDIAVEWESNGQPENNYKTTPPVLDSDGSFFLYSKLTVDKSRWQQGNVFSCSVMHEALHNHYTQKSLSLSPGK

SEQ ID NO: 17 - protein, 452 aa, Mus musculus
RVQPTESIVRFPNITNLCPFGEVFNATRFASVYAWNRKRISNCVADYSVLYNSASFSTFKCYGVSPTKLNDLCFTNVYADSFVIRGDEVRQIAPGQTGKIADYNYKLPDDFTGCVIAWNSNNLDSKVGGNYNYLYRLFRKSNLKPFERDISTEIYQAGSTPCNGVEGFNCYFPLQSYGFQPTNGVGYQPYRVVVLSFELLHAPATVCGPKKSTNLVKNKCVNFFEDKTHTCPPCPAPELLGGPSVFLFPPKPKDTLMISRTPEVTCVVVDVSHEDPEVKFNWYVDGVEVHNAKTKPREEQYNSTYRVVSVLTVLHQDWLNGKEYKCKVSNKALPAPIEKTISKAKGQPREPQVYTLPPCRDELTKNQVSLWCLVKGFYPSDIAVEWESNGQPENNYKTTPPVLDSDGSFFLYSKLTVDKSRWQQGNVFSCSVMHEALHNHYTQKSLSLSPGK

SEQ ID NO: 18 - protein, 555 aa, Mus musculus
DTICIGYHANNSTDTVDTVLEKNVTVTHSVNLLEDSHNGKLCRLKGIAPLQLGKCNIAGWLLGNPECDPLLPVRSWSYIVETPNSENGICYPGDFIDYEELREQLSSVSSFERFEIFPKESSWPNHNTNGVTAACSHEGKSSFYRNLLWLTEKEGSYPKLKNSYVNKKGKEVLVLWGIHHPPNSKEQQNLYQNENAYVSVVTSNYNRRFTPEIAERPKVRDQAGRMNYYWTLLKPGDTIIFEANGNLIAPMYAFALSRGFGSGIITSNASMHECNTKCQTPLGAINSSLPYQNIHPVTIGECPKYVRSAKLRMVTGLRNNPSIQSRFEDKTHTCPPCPAPELLGGPSVFLFPPKPKDTLMISRTPEVTCVVVDVSHEDPEVKFNWYVDGVEVHNAKTKPREEQYNSTYRVVSVLTVLHQDWLNGKEYKCKVSNKALPAPIEKTISKAKGQPREPQVYTLPPCRDELTKNQVSLWCLVKGFYPSDIAVEWESNGQPENNYKTTPPVLDSDGSFFLYSKLTVDKSRWQQGNVFSCSVMHEALHNHYTQKSLSLSPGK

SEQ ID NO: 19 - protein, 327 aa, Mus musculus
MHGDTPTLHEYMLDLQPETTDLYCYEQLNDSSEEEDEIDGPAGQAEPDRAHYNIVTFCCKCDSTLRLCVQSTHVDIRTLEDLLMGTLGIVCPICSQKPFEDKTHTCPPCPAPELLGGPSVFLFPPKPKDTLMISRTPEVTCVVVDVSHEDPEVKFNWYVDGVEVHNAKTKPREEQYNSTYRVVSVLTVLHQDWLNGKEYKCKVSNKALPAPIEKTISKAKGQPREPQVYTLPPCRDELTKNQVSLWCLVKGFYPSDIAVEWESNGQPENNYKTTPPVLDSDGSFFLYSKLTVDKSRWQQGNVFSCSVMHEALHNHYTQKSLSLSPGK

SEQ ID NO: 20 - protein, 241 aa, Homo sapiens
DIQMTQSPSSLSASVGDRVTITCRASQDVSTAVAWYQQKPGKAPKLLIYSASFLYSGVPSRFSGSGSGTDFTLTISSLQPEDFATYYCQQYLYHPATFGQGTKVEIKRGGGGSGGGGSGGGGSEVQLVESGGGLVQPGGSLRLSCAASGFTFSDSWIHWVRQAPGKGLEWVAWISPYGGSTYYADSVKGRFTISADTSKNTAYLQMNSLRAEDTAVYYCARRHWPGGFDYWGQGTLVTVSA

SEQ ID NO: 21 - protein, 165 aa, Homo sapiens [sequence omitted]

SEQ ID NO: 22 - protein, 165 aa, Homo sapiens
CDLPQTHSLGSRRTLMLLAQMRRISLFSCLKDRHDFGFPQEEFGNQFQKAETIPVLHEMIQQIFNLFSTKDSSAAWDETLLDKFYTELYQQLNDLEACVIQGVGVTETPLMKEDSILAVRKYFRRITLYLKEKKYSPCAWEVVRAEIMRSFSLSTNLQESLRSKE

SEQ ID NO: 23 - protein, 227 aa, Homo sapiens
DKTHTCPPCPAPELLGGPSVFLFPPKPKDTLMISRTPEVTCVVVDVSHEDPEVKFNWYVDGVEVHNAKTKPREEQYNSTYRVVSVLTVLHQDWLNGKEYKCKVSNKALPAPIEKTISKAKGQPREPQVCTLPPSRDELTKNQVSLSCAVKGFYPSDIAVEWESNGQPENNYKTTPPVLDSDGSFFLVSKLTVDKSRWQQGNVFSCSVMHEALHNHYTQKSLSLSPGK

SEQ ID NO: 24 - protein, 227 aa, Homo sapiens
DKTHTCPPCPAPELLGGPSVFLFPPKPKDTLMISRTPEVTCVVVDVSHEDPEVKFNWYVDGVEVHNAKTKPREEQYNSTYRVVSVLTVLHQDWLNGKEYKCKVSNKALPAPIEKTISKAKGQPREPQVYTLPPCRDELTKNQVSLWCLVKGFYPSDIAVEWESNGQPENNYKTTPPVLDSDGSFFLYSKLTVDKSRWQQGNVFSCSVMHEALHNHYTQKSLSLSPGK

SEQ ID NO: 25 - protein, 6 aa, synthetic construct
  REGION 1..6: note = artificially synthesized sequence
GSGSGS

SEQ ID NO: 26 - protein, 108 aa, HBV
MGQNLSTSNPLGFFPDHQLDPAFRANTANPDWDFNPNKDTWPDANKVGAGAFGLGFTPPHGGLLGWSPQAQGILQTLPANPPPASTNRQTGRQPTPLSPPLRNTHPQA

SEQ ID NO: 27 - protein, 226 aa, HBV
MENITSGLLGPLLVLQAGFFLLTRILTIPQSLDSWWTSLSFLGEAPVCLGQNSQSPTRNHSPTSCPPICPGYRWMCLRRFIIFLFILLLCLIFLLVLLDYQGMLPVCPLIPGSTTTSTGPCKTCTTPAQGNSMFPSCCCTKPTDGNCTCIPIPSSWAFAKYLWEWASVRFSWLSLLVPFVQWFVGLSPTVWLSAIWMIWYWGPSLYSIVCPFTPLLQIFCCLWVFI

SEQ ID NO: 28 - protein, 226 aa, HBV
MENITSGFLGPLLVLQAGFFLLTRILTIPQSLDSWWTSLNFLGGTTVCLGQSSQSPTSNHSPTSCPPTCPGYRWMCLRRFIIFLFILLLCLIFLLVLLDYQGMLPVCPLIPGSSTTSTGPCRTCMTTAQGTSMYPSCCCTKPSDGNCTCIPIPSSWAFGKFLWEWASARFSWLSLLVPFVQWFVGLSPTVWLSVIWMMWYWGPSLYSILSPFLPLLPIFFCLWVYI

SEQ ID NO: 29 - protein, 534 aa, Mus musculus
CDLPHTYNLGNKRALTVLEEMRRLPPLSCLKDRKDFGFPLEKVDNQQIQKAQAILVLRDLTQQILNLFTSKDLSATWNATLLDSFCNDLHQQLNDLKACVMQEPPLTQEDSLLAVRTYFHRITVYLRKKKHSLCAWEVIRAEVWRALSSSTNLLARLSEEKEGGGGSGGGGSGGGGSRTAKFVAAWTLKAAAGSGSGSMGQNLSTSNPLGFFPDHQLDPAFRANTANPDWDFNPNKDTWPDANKVGAGAFGLGFTPPHGGLLGWSPQAQGILQTLPANPPPASTNRQTGRQPTPLSPPLRNTHPQAFEDKTHTCPPCPAPELLGGPSVFLFPPKPKDQLMISRTPEVTCVVVDVSHEDPEVKFNWYVDGVEVHNAKTKPREEQYNSTYRVVSVLTVLHQDWLNGKEYKCKVSNKALPAPIEKTISKAKGQPREPQVYTLPPSRDELTKNQVSLTCLVKGFYPSDIAVEWESNGQPENNYKTTPPVLDSDGSFLYSKLTVDKSRWQQGNVFSCSVLHEALHNHYTQKSLSLSPGK

SEQ ID NO: 30 - protein, 649 aa, Mus musculus
CDLPHTYNLGNKRALTVLEEMRRLPPLSCLKDRKDFGFPLEKVDNQQIQKAQAILVLRDLTQQILNLFTSKDLSATWNATLLDSFCNDLHQQLNDLKACVMQEPPLTQEDSLLAVRTYFHRITVYLRKKKHSLCAWEVIRAEVWRALSSSTNLLARLSEEKEGGGGSGGGGSGGGGSRTAKFVAAWTLKAAAGSGSGSRVQPTESIVRFPNITNLCPFGEVFNATRFASVYAWNRKRISNCVADYSVLYNSASFSTFKCYGVSPTKLNDLCFTNVYADSFVIRGDEVRQIAPGQTGKIADYNYKLPDDFTGCVIAWNSNNLDSKVGGNYNYLYRLFRKSNLKPFERDISTEIYQAGSTPCNGVEGFNCYFPLQSYGFQPTNGVGYQPYRVVVLSFELLHAPATVCGPKKSTNLVKNKCVNFFEDKTHTCPPCPAPELLGGPSVFLFPPKPKDQLMISRTPEVTCVVVDVSHEDPEVKFNWYVDGVEVHNAKTKPREEQYNSTYRVVSVLTVLHQDWLNGKEYKCKVSNKALPAPIEKTISKAKGQPREPQVYTLPPSRDELTKNQVSLTCLVKGFYPSDIAVEWESNGQPENNYKTTPPVLDSDGSFLYSKLTVDKSRWQQGNVFSCSVLHEALHNHYTQKSLSLSPGK

SEQ ID NO: 31 - protein, 752 aa, Mus musculus
CDLPHTYNLGNKRALTVLEEMRRLPPLSCLKDRKDFGFPLEKVDNQQIQKAQAILVLRDLTQQILNLFTSKDLSATWNATLLDSFCNDLHQQLNDLKACVMQEPPLTQEDSLLAVRTYFHRITVYLRKKKHSLCAWEVIRAEVWRALSSSTNLLARLSEEKEGGGGSGGGGSGGGGSRTAKFVAAWTLKAAAGSGSGSDTICIGYHANNSTDTVDTVLEKNVTVTHSVNLLEDSHNGKLCRLKGIAPLQLGKCNIAGWLLGNPECDPLLPVRSWSYIVETPNSENGICYPGDFIDYEELREQLSSVSSFERFEIFPKESSWPNHNTNGVTAACSHEGKSSFYRNLLWLTEKEGSYPKLKNSYVNKKGKEVLVLWGIHHPPNSKEQQNLYQNENAYVSVVTSNYNRRFTPEIAERPKVRDQAGRMNYYWTLLKPGDTIIFEANGNLIAPMYAFALSRGFGSGIITSNASMHECNTKCQTPLGAINSSLPYQNIHPVTIGECPKYVRSAKLRMVTGLRNNPSIQSRFEDKTHTCPPCPAPELLGGPSVFLFPPKPKDQLMISRTPEVTCVVVDVSHEDPEVKFNWYVDGVEVHNAKTKPREEQYNSTYRVVSVLTVLHQDWLNGKEYKCKVSNKALPAPIEKTISKAKGQPREPQVYTLPPSRDELTKNQVSLTCLVKGFYPSDIAVEWESNGQPENNYKTTPPVLDSDGSFLYSKLTVDKSRWQQGNVFSCSVLHEALHNHYTQKSLSLSPGK

SEQ ID NO: 32 - protein, 524 aa, Mus musculus
CDLPHTYNLGNKRALTVLEEMRRLPPLSCLKDRKDFGFPLEKVDNQQIQKAQAILVLRDLTQQILNLFTSKDLSATWNATLLDSFCNDLHQQLNDLKACVMQEPPLTQEDSLLAVRTYFHRITVYLRKKKHSLCAWEVIRAEVWRALSSSTNLLARLSEEKEGGGGSGGGGSGGGGSRTAKFVAAWTLKAAAGSGSGSMHGDTPTLHEYMLDLQPETTDLYCYEQLNDSSEEEDEIDGPAGQAEPDRAHYNIVTFCCKCDSTLRLCVQSTHVDIRTLEDLLMGTLGIVCPICSQKPFEDKTHTCPPCPAPELLGGPSVFLFPPKPKDQLMISRTPEVTCVVVDVSHEDPEVKFNWYVDGVEVHNAKTKPREEQYNSTYRVVSVLTVLHQDWLNGKEYKCKVSNKALPAPIEKTISKAKGQPREPQVYTLPPSRDELTKNQVSLTCLVKGFYPSDIAVEWESNGQPENNYKTTPPVLDSDGSFLYSKLTVDKSRWQQGNVFSCSVLHEALHNHYTQKSLSLSPGK

SEQ ID NO: 33 - protein, 411 aa, Mus musculus; identical to SEQ ID NO: 15

SEQ ID NO: 34 - protein, 356 aa, Mus musculus
AKFVAAWTLKAAAGSGSGSMGQNLSTSNPLGFFPDHQLDPAFRANTANPDWDFNPNKDTWPDANKVGAGAFGLGFTPPHGGLLGWSPQAQGILQTLPANPPPASTNRQTGRQPTPLSPPLRNTHPQAFEDKTHTCPPCPAPELLGGPSVFLFPPKPKDTLMISRTPEVTCVVVDVSHEDPEVKFNWYVDGVEVHNAKTKPREEQYNSTYRVVSVLTVLHQDWLNGKEYKCKVSNKALPAPIEKTISKAKGQPREPQVYTLPPCRDELTKNQVSLWCLVKGFYPSDIAVEWESNGQPENNYKTTPPVLDSDGSFFLYSKLTVDKSRWQQGNVFSCSVMHEALHNHYTQKSLSLSPGK

SEQ ID NO: 35 - protein, 471 aa, Mus musculus
AKFVAAWTLKAAAGSGSGSRVQPTESIVRFPNITNLCPFGEVFNATRFASVYAWNRKRISNCVADYSVLYNSASFSTFKCYGVSPTKLNDLCFTNVYADSFVIRGDEVRQIAPGQTGKIADYNYKLPDDFTGCVIAWNSNNLDSKVGGNYNYLYRLFRKSNLKPFERDISTEIYQAGSTPCNGVEGFNCYFPLQSYGFQPTNGVGYQPYRVVVLSFELLHAPATVCGPKKSTNLVKNKCVNFFEDKTHTCPPCPAPELLGGPSVFLFPPKPKDTLMISRTPEVTCVVVDVSHEDPEVKFNWYVDGVEVHNAKTKPREEQYNSTYRVVSVLTVLHQDWLNGKEYKCKVSNKALPAPIEKTISKAKGQPREPQVYTLPPCRDELTKNQVSLWCLVKGFYPSDIAVEWESNGQPENNYKTTPPVLDSDGSFFLYSKLTVDKSRWQQGNVFSCSVMHEALHNHYTQKSLSLSPGK

SEQ ID NO: 36 - protein, 574 aa, Mus musculus
AKFVAAWTLKAAAGSGSGSDTICIGYHANNSTDTVDTVLEKNVTVTHSVNLLEDSHNGKLCRLKGIAPLQLGKCNIAGWLLGNPECDPLLPVRSWSYIVETPNSENGICYPGDFIDYEELREQLSSVSSFERFEIFPKESSWPNHNTNGVTAACSHEGKSSFYRNLLWLTEKEGSYPKLKNSYVNKKGKEVLVLWGIHHPPNSKEQQNLYQNENAYVSVVTSNYNRRFTPEIAERPKVRDQAGRMNYYWTLLKPGDTIIFEANGNLIAPMYAFALSRGFGSGIITSNASMHECNTKCQTPLGAINSSLPYQNIHPVTIGECPKYVRSAKLRMVTGLRNNPSIQSRFEDKTHTCPPCPAPELLGGPSVFLFPPKPKDTLMISRTPEVTCVVVDVSHEDPEVKFNWYVDGVEVHNAKTKPREEQYNSTYRVVSVLTVLHQDWLNGKEYKCKVSNKALPAPIEKTISKAKGQPREPQVYTLPPCRDELTKNQVSLWCLVKGFYPSDIAVEWESNGQPENNYKTTPPVLDSDGSFFLYSKLTVDKSRWQQGNVFSCSVMHEALHNHYTQKSLSLSPGK

SEQ ID NO: 37 - protein, 346 aa, Mus musculus
AKFVAAWTLKAAAGSGSGSMHGDTPTLHEYMLDLQPETTDLYCYEQLNDSSEEEDEIDGPAGQAEPDRAHYNIVTFCCKCDSTLRLCVQSTHVDIRTLEDLLMGTLGIVCPICSQKPFEDKTHTCPPCPAPELLGGPSVFLFPPKPKDTLMISRTPEVTCVVVDVSHEDPEVKFNWYVDGVEVHNAKTKPREEQYNSTYRVVSVLTVLHQDWLNGKEYKCKVSNKALPAPIEKTISKAKGQPREPQVYTLPPCRDELTKNQVSLWCLVKGFYPSDIAVEWESNGQPENNYKTTPPVLDSDGSFFLYSKLTVDKSRWQQGNVFSCSVMHEALHNHYTQKSLSLSPGK

SEQ ID NO: 38 - protein, 518 aa, Homo sapiens
CDLPQTHSLGSRRTLMLLAQMRRISLFSCLKDRHDFGFPQEEFGNQFQKAETIPVLHEMIQQIFNLFSTKDSSAAWDETLLDKFYTELYQQLNDLEACVIQGVGVTETPLMKEDSILAVRKYFQRITLYLKEKKYSPCAWEVVRAEIMRSFSLSTNLQESLRSKEGGGGSGGGGSGGGGSRTMGQNLSTSNPLGFFPDHQLDPAFRANTANPDWDFNPNKDTWPDANKVGAGAFGLGFTPPHGGLLGWSPQAQGILQTLPANPPPASTNRQTGRQPTPLSPPLRNTHPQAFEDKTHTCPPCPAPELLGGPSVFLFPPKPKDQLMISRTPEVTCVVVDVSHEDPEVKFNWYVDGVEVHNAKTKPREEQYNSTYRVVSVLTVLHQDWLNGKEYKCKVSNKALPAPIEKTISKAKGQPREPQVYTLPPSRDELTKNQVSLTCLVKGFYPSDIAVEWESNGQPENNYKTTPPVLDSDGSFLYSKLTVDKSRWQQGNVFSCSVLHEALHNHYTQKSLSLSPGK

SEQ ID NO: 39 - protein, 633 aa, Homo sapiens
CDLPQTHSLGSRRTLMLLAQMRRISLFSCLKDRHDFGFPQEEFGNQFQKAETIPVLHEMIQQIFNLFSTKDSSAAWDETLLDKFYTELYQQLNDLEACVIQGVGVTETPLMKEDSILAVRKYFQRITLYLKEKKYSPCAWEVVRAEIMRSFSLSTNLQESLRSKEGGGGSGGGGSGGGGSRTRVQPTESIVRFPNITNLCPFGEVFNATRFASVYAWNRKRISNCVADYSVLYNSASFSTFKCYGVSPTKLNDLCFTNVYADSFVIRGDEVRQIAPGQTGKIADYNYKLPDDFTGCVIAWNSNNLDSKVGGNYNYLYRLFRKSNLKPFERDISTEIYQAGSTPCNGVEGFNCYFPLQSYGFQPTNGVGYQPYRVVVLSFELLHAPATVCGPKKSTNLVKNKCVNFFEDKTHTCPPCPAPELLGGPSVFLFPPKPKDQLMISRTPEVTCVVVDVSHEDPEVKFNWYVDGVEVHNAKTKPREEQYNSTYRVVSVLTVLHQDWLNGKEYKCKVSNKALPAPIEKTISKAKGQPREPQVYTLPPSRDELTKNQVSLTCLVKGFYPSDIAVEWESNGQPENNYKTTPPVLDSDGSFLYSKLTVDKSRWQQGNVFSCSVLHEALHNHYTQKSLSLSPGK

SEQ ID NO: 40 - protein, 736 aa, Homo sapiens
CDLPQTHSLGSRRTLMLLAQMRRISLFSCLKDRHDFGFPQEEFGNQFQKAETIPVLHEMIQQIFNLFSTKDSSAAWDETLLDKFYTELYQQLNDLEACVIQGVGVTETPLMKEDSILAVRKYFQRITLYLKEKKYSPCAWEVVRAEIMRSFSLSTNLQESLRSKEGGGGSGGGGSGGGGSRTDTICIGYHANNSTDTVDTVLEKNVTVTHSVNLLEDSHNGKLCRLKGIAPLQLGKCNIAGWLLGNPECDPLLPVRSWSYIVETPNSENGICYPGDFIDYEELREQLSSVSSFERFEIFPKESSWPNHNTNGVTAACSHEGKSSFYRNLLWLTEKEGSYPKLKNSYVNKKGKEVLVLWGIHHPPNSKEQQNLYQNENAYVSVVTSNYNRRFTPEIAERPKVRDQAGRMNYYWTLLKPGDTIIFEANGNLIAPMYAFALSRGFGSGIITSNASMHECNTKCQTPLGAINSSLPYQNIHPVTIGECPKYVRSAKLRMVTGLRNNPSIQSRFEDKTHTCPPCPAPELLGGPSVFLFPPKPKDQLMISRTPEVTCVVVDVSHEDPEVKFNWYVDGVEVHNAKTKPREEQYNSTYRVVSVLTVLHQDWLNGKEYKCKVSNKALPAPIEKTISKAKGQPREPQVYTLPPSRDELTKNQVSLTCLVKGFYPSDIAVEWESNGQPENNYKTTPPVLDSDGSFLYSKLTVDKSRWQQGNVFSCSVLHEALHNHYTQKSLSLSPGK

SEQ ID NO: 41 - protein, 508 aa, Homo sapiens
CDLPQTHSLGSRRTLMLLAQMRRISLFSCLKDRHDFGFPQEEFGNQFQKAETIPVLHEMIQQIFNLFSTKDSSAAWDETLLDKFYTELYQQLNDLEACVIQGVGVTETPLMKEDSILAVRKYFQRITLYLKEKKYSPCAWEVVRAEIMRSFSLSTNLQESLRSKEGGGGSGGGGSGGGGSRTMHGDTPTLHEYMLDLQPETTDLYCYEQLNDSSEEEDEIDGPAGQAEPDRAHYNIVTFCCKCDSTLRLCVQSTHVDIRTLEDLLMGTLGIVCPICSQKPFEDKTHTCPPCPAPELLGGPSVFLFPPKPKDQLMISRTPEVTCVVVDVSHEDPEVKFNWYVDGVEVHNAKTKPREEQYNSTYRVVSVLTVLHQDWLNGKEYKCKVSNKALPAPIEKTISKAKGQPREPQVYTLPPSRDELTKNQVSLTCLVKGFYPSDIAVEWESNGQPENNYKTTPPVLDSDGSFLYSKLTVDKSRWQQGNVFSCSVLHEALHNHYTQKSLSLSPGK

SEQ ID NO: 42 - protein, 414 aa, Homo sapiens
CDLPQTHSLGSRRTLMLLAQMRRISLFSCLKDRHDFGFPQEEFGNQFQKAETIPVLHEMIQQIFNLFSTKDSSAAWDETLLDKFYTELYQQLNDLEACVIQGVGVTETPLMKEDSILAVRKYFQRITLYLKEKKYSPCAWEVVRAEIMRSFSLSTNLQESLRSKESGGGGSGGGGSGGGGSGGGGRTDKTHTCPPCPAPELLGGPSVFLFPPKPKDTLMISRTPEVTCVVVDVSHEDPEVKFNWYVDGVEVHNAKTKPREEQYNSTYRVVSVLTVLHQDWLNGKEYKCKVSNKALPAPIEKTISKAKGQPREPQVCTLPPSRDELTKNQVSLSCAVKGFYPSDIAVEWESNGQPENNYKTTPPVLDSDGSFKLVSKLTVDKSRWQQGNVFSCSVMHEALHNHYTQKSLSLSPGK

SEQ ID NO: 43 - protein, 337 aa, Homo sapiens
MGQNLSTSNPLGFFPDHQLDPAFRANTANPDWDFNPNKDTWPDANKVGAGAFGLGFTPPHGGLLGWSPQAQGILQTLPANPPPASTNRQTGRQPTPLSPPLRNTHPQAFEDKTHTCPPCPAPELLGGPSVFLFPPKPKDTLMISRTPEVTCVVVDVSHEDPEVKFNWYVDGVEVHNAKTKPREEQYNSTYRVVSVLTVLHQDWLNGKEYKCKVSNKALPAPIEKTISKAKGQPREPQVCTLPPSRDELTKNQVSLSCAVKGFYPSDIAVEWESNGQPENNYKTTPPVLDSDGSFFLVSKLTVDKSRWQQGNVFSCSVMHEALHNHYTQKSLSLSPGK

SEQ ID NO: 44 - protein, 452 aa, Homo sapiens; identical to SEQ ID NO: 17

SEQ ID NO: 45 - protein, 555 aa, Homo sapiens; identical to SEQ ID NO: 18

SEQ ID NO: 46 - protein, 327 aa, Homo sapiens; identical to SEQ ID NO: 19

SEQ ID NO: 47 - protein, 520 aa, Homo sapiens
CDLPQTHSLGSRRTLMLLAQMRRISLFSCLKDRHDFGFPQEEFGNQFQKAETIPVLHEMIQQIFNLFSTKDSSAAWDETLLDKFYTELYQQLNDLEACVIQGVGVTETPLMKEDSILAVRKYFQRITLYLKEKKYSPCAWEVVRAEIMRSFSLSTNLQESLRSKEAKFVAAWTLKAAAGSGSGSMGQNLSTSNPLGFFPDHQLDPAFRANTANPDWDFNPNKDTWPDANKVGAGAFGLGFTPPHGGLLGWSPQAQGILQTLPANPPPASTNRQTGRQPTPLSPPLRNTHPQAFEDKTHTCPPCPAPELLGGPSVFLFPPKPKDQLMISRTPEVTCVVVDVSHEDPEVKFNWYVDGVEVHNAKTKPREEQYNSTYRVVSVLTVLHQDWLNGKEYKCKVSNKALPAPIEKTISKAKGQPREPQVYTLPPSRDELTKNQVSLTCLVKGFYPSDIAVEWESNGQPENNYKTTPPVLDSDGSFLYSKLTVDKSRWQQGNVFSCSVLHEALHNHYTQKSLSLSPGK

SEQ ID NO: 48 - protein, 635 aa, Homo sapiens
CDLPQTHSLGSRRTLMLLAQMRRISLFSCLKDRHDFGFPQEEFGNQFQKAETIPVLHEMIQQIFNLFSTKDSSAAWDETLLDKFYTELYQQLNDLEACVIQGVGVTETPLMKEDSILAVRKYFQRITLYLKEKKYSPCAWEVVRAEIMRSFSLSTNLQESLRSKEAKFVAAWTLKAAAGSGSGSRVQPTESIVRFPNITNLCPFGEVFNATRFASVYAWNRKRISNCVADYSVLYNSASFSTFKCYGVSPTKLNDLCFTNVYADSFVIRGDEVRQIAPGQTGKIADYNYKLPDDFTGCVIAWNSNNLDSKVGGNYNYLYRLFRKSNLKPFERDISTEIYQAGSTPCNGVEGFNCYFPLQSYGFQPTNGVGYQPYRVVVLSFELLHAPATVCGPKKSTNLVKNKCVNFFEDKTHTCPPCPAPELLGGPSVFLFPPKPKDQLMISRTPEVTCVVVDVSHEDPEVKFNWYVDGVEVHNAKTKPREEQYNSTYRVVSVLTVLHQDWLNGKEYKCKVSNKALPAPIEKTISKAKGQPREPQVYTLPPSRDELTKNQVSLTCLVKGFYPSDIAVEWESNGQPENNYKTTPPVLDSDGSFLYSKLTVDKSRWQQGNVFSCSVLHEALHNHYTQKSLSLSPGK

SEQ ID NO: 49 - protein, 738 aa, Homo sapiens
CDLPQTHSLGSRRTLMLLAQMRRISLFSCLKDRHDFGFPQEEFGNQFQKAETIPVLHEMIQQIFNLFSTKDSSAAWDETLLDKFYTELYQQLNDLEACVIQGVGVTETPLMKEDSILAVRKYFQRITLYLKEKKYSPCAWEVVRAEIMRSFSLSTNLQESLRSKEAKFVAAWTLKAAAGSGSGSDTICIGYHANNSTDTVDTVLEKNVTVTHSVNLLEDSHNGKLCRLKGIAPLQLGKCNIAGWLLGNPECDPLLPVRSWSYIVETPNSENGICYPGDFIDYEELREQLSSVSSFERFEIFPKESSWPNHNTNGVTAACSHEGKSSFYRNLLWLTEKEGSYPKLKNSYVNKKGKEVLVLWGIHHPPNSKEQQNLYQNENAYVSVVTSNYNRRFTPEIAERPKVRDQAGRMNYYWTLLKPGDTIIFEANGNLIAPMYAFALSRGFGSGIITSNASMHECNTKCQTPLGAINSSLPYQNIHPVTIGECPKYVRSAKLRMVTGLRNNPSIQSRFEDKTHTCPPCPAPELLGGPSVFLFPPKPKDQLMISRTPEVTCVVVDVSHEDPEVKFNWYVDGVEVHNAKTKPREEQYNSTYRVVSVLTVLHQDWLNGKEYKCKVSNKALPAPIEKTISKAKGQPREPQVYTLPPSRDELTKNQVSLTCLVKGFYPSDIAVEWESNGQPENNYKTTPPVLDSDGSFLYSKLTVDKSRWQQGNVFSCSVLHEALHNHYTQKSLSLSPGK

SEQ ID NO: 50 - protein, 510 aa, Homo sapiens
CDLPQTHSLGSRRTLMLLAQMRRISLFSCLKDRHDFGFPQEEFGNQFQKAETIPVLHEMIQQIFNLFSTKDSSAAWDETLLDKFYTELYQQLNDLEACVIQGVGVTETPLMKEDSILAVRKYFQRITLYLKEKKYSPCAWEVVRAEIMRSFSLSTNLQESLRSKEAKFVAAWTLKAAAGSGSGSMHGDTPTLHEYMLDLQPETTDLYCYEQLNDSSEEEDEIDGPAGQAEPDRAHYNIVTFCCKCDSTLRLCVQSTHVDIRTLEDLLMGTLGIVCPICSQKPFEDKTHTCPPCPAPELLGGPSVFLFPPKPKDQLMISRTPEVTCVVVDVSHEDPEVKFNWYVDGVEVHNAKTKPREEQYNSTYRVVSVLTVLHQDWLNGKEYKCKVSNKALPAPIEKTISKAKGQPREPQVYTLPPSRDELTKNQVSLTCLVKGFYPSDIAVEWESNGQPENNYKTTPPVLDSDGSFLYSKLTVDKSRWQQGNVFSCSVLHEALHNHYTQKSLSLSPGK

SEQ ID NO: 51 - protein, 414 aa, Homo sapiens
CDLPQTHSLGSRRTLMLLAQMRRISLFSCLKDRHDFGFPQEEFGNQFQKAETIPVLHEMIQQIFNLFSTKDSSAAWDETLLDKFYTELYQQLNDLEACVIQGVGVTETPLMKEDSILAVRKYFQRITLYLKEKKYSPCAWEVVRAEIMRSFSLSTNLQESLRSKESGGGGSGGGGSGGGGSGGGGRTDKTHTCPPCPAPELLGGPSVFLFPPKPKDTLMISRTPEVTCVVVDVSHEDPEVKFNWYVDGVEVHNAKTKPREEQYNSTYRVVSVLTVLHQDWLNGKEYKCKVSNKALPAPIEKTISKAKGQPREPQVCTLPPSRDELTKNQVSLSCAVKGFYPSDIAVEWESNGQPENNYKTTPPVLDSDGSFFLVSKLTVDKSRWQQGNVFSCSVMHEALHNHYTQKSLSLSPGK

SEQ ID NO: 52 - protein, 356 aa, Homo sapiens; identical to SEQ ID NO: 34

SEQ ID NO: 53 - protein, 471 aa, Homo sapiens; identical to SEQ ID NO: 35

SEQ ID NO: 54 - protein, 574 aa, Homo sapiens; identical to SEQ ID NO: 36

SEQ ID NO: 55 - protein, 346 aa, Homo sapiens; identical to SEQ ID NO: 37

SEQ ID NO: 56 - protein, 518 aa, Homo sapiens
CDLPQTHSLGSRRTLMLLAQMRRISLFSCLKDRHDFGFPQEEFGNQFQKAETIPVLHEMIQQIFNLFSTKDSSAAWDETLLDKFYTELYQQLNDLEACVIQGVGVTETPLMKEDSILAVRKYFRRITLYLKEKKYSPCAWEVVRAEIMRSFSLSTNLQESLRSKEGGGGSGGGGSGGGGSRTMGQNLSTSNPLGFFPDHQLDPAFRANTANPDWDFNPNKDTWPDANKVGAGAFGLGFTPPHGGLLGWSPQAQGILQTLPANPPPASTNRQTGRQPTPLSPPLRNTHPQAFEDKTHTCPPCPAPELLGGPSVFLFPPKPKDQLMISRTPEVTCVVVDVSHEDPEVKFNWYVDGVEVHNAKTKPREEQYNSTYRVVSVLTVLHQDWLNGKEYKCKVSNKALPAPIEKTISKAKGQPREPQVYTLPPSRDELTKNQVSLTCLVKGFYPSDIAVEWESNGQPENNYKTTPPVLDSDGSFLYSKLTVDKSRWQQGNVFSCSVLHEALHNHYTQKSLSLSPGK

SEQ ID NO: 57 - protein, 633 aa, Homo sapiens
CDLPQTHSLGSRRTLMLLAQMRRISLFSCLKDRHDFGFPQEEFGNQFQKAETIPVLHEMIQQIFNLFSTKDSSAAWDETLLDKFYTELYQQLNDLEACVIQGVGVTETPLMKEDSILAVRKYFRRITLYLKEKKYSPCAWEVVRAEIMRSFSLSTNLQESLRSKEGGGGSGGGGSGGGGSRTRVQPTESIVRFPNITNLCPFGEVFNATRFASVYAWNRKRISNCVADYSVLYNSASFSTFKCYGVSPTKLNDLCFTNVYADSFVIRGDEVRQIAPGQTGKIADYNYKLPDDFTGCVIAWNSNNLDSKVGGNYNYLYRLFRKSNLKPFERDISTEIYQAGSTPCNGVEGFNCYFPLQSYGFQPTNGVGYQPYRVVVLSFELLHAPATVCGPKKSTNLVKNKCVNFFEDKTHTCPPCPAPELLGGPSVFLFPPKPKDQLMISRTPEVTCVVVDVSHEDPEVKFNWYVDGVEVHNAKTKPREEQYNSTYRVVSVLTVLHQDWLNGKEYKCKVSNKALPAPIEKTISKAKGQPREPQVYTLPPSRDELTKNQVSLTCLVKGFYPSDIAVEWESNGQPENNYKTTPPVLDSDGSFLYSKLTVDKSRWQQGNVFSCSVLHEALHNHYTQKSLSLSPGK

SEQ ID NO: 58 - protein, 736 aa, Homo sapiens
CDLPQTHSLGSRRTLMLLAQMRRISLFSCLKDRHDFGFPQEEFGNQFQKAETIPVLHEMIQQIFNLFSTKDSSAAWDETLLDKFYTELYQQLNDLEACVIQGVGVTETPLMKEDSILAVRKYFRRITLYLKEKKYSPCAWEVVRAEIMRSFSLSTNLQESLRSKEGGGGSGGGGSGGGGSRTDTICIGYHANNSTDTVDTVLEKNVTVTHSVNLLEDSHNGKLCRLKGIAPLQLGKCNIAGWLLGNPECDPLLPVRSWSYIVETPNSENGICYPGDFIDYEELREQLSSVSSFERFEIFPKESSWPNHNTNGVTAACSHEGKSSFYRNLLWLTEKEGSYPKLKNSYVNKKGKEVLVLWGIHHPPNSKEQQNLYQNENAYVSVVTSNYNRRFTPEIAERPKVRDQAGRMNYYWTLLKPGDTIIFEANGNLIAPMYAFALSRGFGSGIITSNASMHECNTKCQTPLGAINSSLPYQNIHPVTIGECPKYVRSAKLRMVTGLRNNPSIQSRFEDKTHTCPPCPAPELLGGPSVFLFPPKPKDQLMISRTPEVTCVVVDVSHEDPEVKFNWYVDGVEVHNAKTKPREEQYNSTYRVVSVLTVLHQDWLNGKEYKCKVSNKALPAPIEKTISKAKGQPREPQVYTLPPSRDELTKNQVSLTCLVKGFYPSDIAVEWESNGQPENNYKTTPPVLDSDGSFLYSKLTVDKSRWQQGNVFSCSVLHEALHNHYTQKSLSLSPGK

SEQ ID NO: 59 - protein, 508 aa, Homo sapiens
CDLPQTHSLGSRRTLMLLAQMRRISLFSCLKDRHDFGFPQEEFGNQFQKAETIPVLHEMIQQIFNLFSTKDSSAAWDETLLDKFYTELYQQLNDLEACVIQGVGVTETPLMKEDSILAVRKYFRRITLYLKEKKYSPCAWEVVRAEIMRSFSLSTNLQESLRSKEGGGGSGGGGSGGGGSRTMHGDTPTLHEYMLDLQPETTDLYCYEQLNDSSEEEDEIDGPAGQAEPDRAHYNIVTFCCKCDSTLRLCVQSTHVDIRTLEDLLMGTLGIVCPICSQKPFEDKTHTCPPCPAPELLGGPSVFLFPPKPKDQLMISRTPEVTCVVVDVSHEDPEVKFNWYVDGVEVHNAKTKPREEQYNSTYRVVSVLTVLHQDWLNGKEYKCKVSNKALPAPIEKTISKAKGQPREPQVYTLPPSRDELTKNQVSLTCLVKGFYPSDIAVEWESNGQPENNYKTTPPVLDSDGSFLYSKLTVDKSRWQQGNVFSCSVLHEALHNHYTQKSLSLSPGK

SEQ ID NO: 60 - protein, 414 aa, Homo sapiens
CDLPQTHSLGSRRTLMLLAQMRRISLFSCLKDRHDFGFPQEEFGNQFQKAETIPVLHEMIQQIFNLFSTKDSSAAWDETLLDKFYTELYQQLNDLEACVIQGVGVTETPLMKEDSILAVRKYFRRITLYLKEKKYSPCAWEVVRAEIMRSFSLSTNLQESLRSKESGGGGSGGGGSGGGGSGGGGRTDKTHTCPPCPAPELLGGPSVFLFPPKPKDTLMISRTPEVTCVVVDVSHEDPEVKFNWYVDGVEVHNAKTKPREEQYNSTYRVVSVLTVLHQDWLNGKEYKCKVSNKALPAPIEKTISKAKGQPREPQVCTLPPSRDELTKNQVSLSCAVKGFYPSDIAVEWESNGQPENNYKTTPPVLDSDGSFFLVSKLTVDKSRWQQGNVFSCSVMHEALHNHYTQKSLSLSPGK

SEQ ID NO: 61 - protein, 337 aa, Homo sapiens; identical to SEQ ID NO: 16

SEQ ID NO: 62 - protein, 452 aa, Homo sapiens; identical to SEQ ID NO: 17

SEQ ID NO: 63 - protein, 555 aa, Homo sapiens; identical to SEQ ID NO: 18

SEQ ID NO: 64 - protein, 327 aa, Homo sapiens; identical to SEQ ID NO: 19

SEQ ID NO: 65 - protein, 520 aa, Homo sapiens
CDLPQTHSLGSRRTLMLLAQMRRISLFSCLKDRHDFGFPQEEFGNQFQKAETIPVLHEMIQQIFNLFSTKDSSAAWDETLLDKFYTELYQQLNDLEACVIQGVGVTETPLMKEDSILAVRKYFRRITLYLKEKKYSPCAWEVVRAEIMRSFSLSTNLQESLRSKEAKFVAAWTLKAAAGSGSGSMGQNLSTSNPLGFFPDHQLDPAFRANTANPDWDFNPNKDTWPDANKVGAGAFGLGFTPPHGGLLGWSPQAQGILQTLPANPPPASTNRQTGRQPTPLSPPLRNTHPQAFEDKTHTCPPCPAPELLGGPSVFLFPPKPKDQLMISRTPEVTCVVVDVSHEDPEVKFNWYVDGVEVHNAKTKPREEQYNSTYRVVSVLTVLHQDWLNGKEYKCKVSNKALPAPIEKTISKAKGQPREPQVYTLPPSRDELTKNQVSLTCLVKGFYPSDIAVEWESNGQPENNYKTTPPVLDSDGSFLYSKLTVDKSRWQQGNVFSCSVLHEALHNHYTQKSLSLSPGK

SEQ ID NO: 66 - protein, 635 aa, Homo sapiens
CDLPQTHSLGSRRTLMLLAQMRRISLFSCLKDRHDFGFPQEEFGNQFQKAETIPVLHEMIQQIFNLFSTKDSSAAWDETLLDKFYTELYQQLNDLEACVIQGVGVTETPLMKEDSILAVRKYFRRITLYLKEKKYSPCAWEVVRAEIMRSFSLSTNLQESLRSKEAKFVAAWTLKAAAGSGSGSRVQPTESIVRFPNITNLCPFGEVFNATRFASVYAWNRKRISNCVADYSVLYNSASFSTFKCYGVSPTKLNDLCFTNVYADSFVIRGDEVRQIAPGQTGKIADYNYKLPDDFTGCVIAWNSNNLDSKVGGNYNYLYRLFRKSNLKPFERDISTEIYQAGSTPCNGVEGFNCYFPLQSYGFQPTNGVGYQPYRVVVLSFELLHAPATVCGPKKSTNLVKNKCVNFFEDKTHTCPPCPAPELLGGPSVFLFPPKPKDQLMISRTPEVTCVVVDVSHEDPEVKFNWYVDGVEVHNAKTKPREEQYNSTYRVVSVLTVLHQDWLNGKEYKCKVSNKALPAPIEKTISKAKGQPREPQVYTLPPSRDELTKNQVSLTCLVKGFYPSDIAVEWESNGQPENNYKTTPPVLDSDGSFLYSKLTVDKSRWQQGNVFSCSVLHEALHNHYTQKSLSLSPGK

SEQ ID NO: 67 - protein, 738 aa, Homo sapiens
CDLPQTHSLGSRRTLMLLAQMRRISLFSCLKDRHDFGFPQEEFGNQFQKAETIPVLHEMIQQIFNLFSTKDSSAAWDETLLDKFYTELYQQLNDLEACVIQGVGVTETPLMKEDSILAVRKYFRRITLYLKEKKYSPCAWEVVRAEIMRSFSLSTNLQESLRSKEAKFVAAWTLKAAAGSGSGSDTICIGYHANNSTDTVDTVLEKNVTVTHSVNLLEDSHNGKLCRLKGIAPLQLGKCNIAGWLLGNPECDPLLPVRSWSYIVETPNSENGICYPGDFIDYEELREQLSSVSSFERFEIFPKESSWPNHNTNGVTAACSHEGKSSFYRNLLWLTEKEGSYPKLKNSYVNKKGKEVLVLWGIHHPPNSKEQQNLYQNENAYVSVVTSNYNRRFTPEIAERPKVRDQAGRMNYYWTLLKPGDTIIFEANGNLIAPMYAFALSRGFGSGIITSNASMHECNTKCQTPLGAINSSLPYQNIHPVTIGECPKYVRSAKLRMVTGLRNNPSIQSRFEDKTHTCPPCPAPELLGGPSVFLFPPKPKDQLMISRTPEVTCVVVDVSHEDPEVKFNWYVDGVEVHNAKTKPREEQYNSTYRVVSVLTVLHQDWLNGKEYKCKVSNKALPAPIEKTISKAKGQPREPQVYTLPPSRDELTKNQVSLTCLVKGFYPSDIAVEWESNGQPENNYKTTPPVLDSDGSFLYSKLTVDKSRWQQGNVFSCSVLHEALHNHYTQKSLSLSPGK

SEQ ID NO: 68 - protein, 510 aa, Homo sapiens
CDLPQTHSLGSRRTLMLLAQMRRISLFSCLKDRHDFGFPQEEFGNQFQKAETIPVLHEMIQQIFNLFSTKDSSAAWDETLLDKFYTELYQQLNDLEACVIQGVGVTETPLMKEDSILAVRKYFRRITLYLKEKKYSPCAWEVVRAEIMRSFSLSTNLQESLRSKEAKFVAAWTLKAAAGSGSGSMHGDTPTLHEYMLDLQPETTDLYCYEQLNDSSEEEDEIDGPAGQAEPDRAHYNIVTFCCKCDSTLRLCVQSTHVDIRTLEDLLMGTLGIVCPICSQKPFEDKTHTCPPCPAPELLGGPSVFLFPPKPKDQLMISRTPEVTCVVVDVSHEDPEVKFNWYVDGVEVHNAKTKPREEQYNSTYRVVSVLTVLHQDWLNGKEYKCKVSNKALPAPIEKTISKAKGQPREPQVYTLPPSRDELTKNQVSLTCLVKGFYPSDIAVEWESNGQPENNYKTTPPVLDSDGSFLYSKLTVDKSRWQQGNVFSCSVLHEALHNHYTQKSLSLSPGK

SEQ ID NO: 69 - protein, 414 aa, Homo sapiens; identical to SEQ ID NO: 60

SEQ ID NO: 70 - protein, 356 aa, Homo sapiens; identical to SEQ ID NO: 34

SEQ ID NO: 71 - protein, 471 aa, Homo sapiens; identical to SEQ ID NO: 35

SEQ ID NO: 72 - protein, 574 aa, Homo sapiens; identical to SEQ ID NO: 36

SEQ ID NO: 73 - protein, 346 aa, Homo sapiens; identical to SEQ ID NO: 37

SEQ ID NO: 74 - protein, 118 aa, Homo sapiens
EVQLVESGGGLVQPGGSLRLSCAASGFTFSDSWIHWVRQAPGKGLEWVAWISPYGGSTYYADSVKGRFTISADTSKNTAYLQMNSLRAEDTAVYYCARRHWPGGFDYWGQGTLVTVSA

SEQ ID NO: 75 - protein, 108 aa, Homo sapiens
DIQMTQSPSSLSASVGDRVTITCRASQDVSTAVAWYQQKPGKAPKLLIYSASFLYSGVPSRFSGSGSGTDFTLTISSLQPEDFATYYCQQYLYHPATFGQGTKVEIKR

SEQ ID NO: 76 - protein, 1258 aa, SARS-CoV-2
VNLTTRTQLPPAYTNSFTRGVYYPDKVFRSSVLHSTQDLFLPFFSNVTWFHAIHVSGTNGTKRFDNPVLPFNDGVYFASTEKSNIIRGWIFGTTLDSKTQSLLIVNNATNVVIKVCEFQFCNDPFLGVYYHKNNKSWMESEFRVYSSANNCTFEYVSQPFLMDLEGKQGNFKNLREFVFKNIDGYFKIYSKHTPINLVRDLPQGFSALEPLVDLPIGINITRFQTLLALHRSYLTPGDSSSGWTAGAAAYYVGYLQPRTFLLKYNENGTITDAVDCALDPLSETKCTLKSFTVEKGIYQTSNFRVQPTESIVRFPNITNLCPFGEVFNATRFASVYAWNRKRISNCVADYSVLYNSASFSTFKCYGVSPTKLNDLCFTNVYADSFVIRGDEVRQIAPGQTGKIADYNYKLPDDFTGCVIAWNSNNLDSKVGGNYNYLYRLFRKSNLKPFERDISTEIYQAGSTPCNGVEGFNCYFPLQSYGFQPTNGVGYQPYRVVVLSFELLHAPATVCGPKKSTNLVKNKCVNFNFNGLTGTGVLTESNKKFLPFQQFGRDIADTTDAVRDPQTLEILDITPCSFGGVSVITPGTNTSNQVAVLYQDVNCTEVPVAIHADQLTPTWRVYSTGSNVFQTRAGCLIGAEHVNNSYECDIPIGAGICASYQTQTNSPRRARSVASQSIIAYTMSLGAENSVAYSNNSIAIPTNFTISVTTEILPVSMTKTSVDCTMYICGDSTECSNLLLQYGSFCTQLNRALTGIAVEQDKNTQEVFAQVKQIYKTPPIKDFGGFNFSQILPDPSKPSKRSFIEDLLFNKVTLADAGFIKQYGDCLGDIAARDLICAQKFNGLTVLPPLLTDEMIAQYTSALLAGTITSGWTFGAGAALQIPFAMQMAYRFNGIGVTQNVLYENQKLIANQFNSAIGKIQDSLSSTASALGKLQDVVNQNAQALNTLVKQLSSNFGAISSVLNDILSRLDKVEAEVQIDRLITGRLQSLQTYVTQQLIRAAEIRASANLAATKMSECVLGQSKRVDFCGKGYHLMSFPQSAPHGVVFLHVTYVPAQEKNFTTAPAICHDGKAHFPREGVFVSNGTHWFVTQRNFYEPQIITTDNTFVSGNCDVVIGIVNNTVYDPLQPELDSFKEELDKYFKNHTSPDVDLGDISGINASVVNIQKEIDRLNEVAKNLNESLIDLQELGKYEQYIKWPWYIWLGFIAGLIAIVMVTIMLCCMTSCCSCLKGCCSCGSCCKFDEDDSEPVLKGVKLHYT

SEQ ID NO: 77 - protein, 670 aa, SARS-CoV-2
VNLTTRTQLPPAYTNSFTRGVYYPDKVFRSSVLHSTQDLFLPFFSNVTWFHAIHVSGTNGTKRFDNPVLPFNDGVYFASTEKSNIIRGWIFGTTLDSKTQSLLIVNNATNVVIKVCEFQFCNDPFLGVYYHKNNKSWMESEFRVYSSANNCTFEYVSQPFLMDLEGKQGNFKNLREFVFKNIDGYFKIYSKHTPINLVRDLPQGFSALEPLVDLPIGINITRFQTLLALHRSYLTPGDSSSGWTAGAAAYYVGYLQPRTFLLKYNENGTITDAVDCALDPLSETKCTLKSFTVEKGIYQTSNFRVQPTESIVRFPNITNLCPFGEVFNATRFASVYAWNRKRISNCVADYSVLYNSASFSTFKCYGVSPTKLNDLCFTNVYADSFVIRGDEVRQIAPGQTGKIADYNYKLPDDFTGCVIAWNSNNLDSKVGGNYNYLYRLFRKSNLKPFERDISTEIYQAGSTPCNGVEGFNCYFPLQSYGFQPTNGVGYQPYRVVVLSFELLHAPATVCGPKKSTNLVKNKCVNFNFNGLTGTGVLTESNKKFLPFQQFGRDIADTTDAVRDPQTLEILDITPCSFGGVSVITPGTNTSNQVAVLYQDVNCTEVPVAIHADQLTPTWRVYSTGSNVFQTRAGCLIGAEHVNNSYECDIPIGAGICASYQTQTNSPRRAR

SEQ ID NO: 78 - protein, 223 aa, SARS-CoV-2; identical to SEQ ID NO: 8

SEQ ID NO: 79 - protein, 223 aa, SARS-CoV-2
RVQPTESIVRFPNITNLCPFGEVFNATRFASVYAWNRKRISNCVADYSVLYNSASFSTFKCYGVSPTKLNDLCFTNVYADSFVIRGDEVRQIAPGQTGKIADYNYKLPDDFTGCVIAWNSNNLDSKVGGNYNYLYRLFRKSNLKPFERDISTEIYQAGSTPCNGVEGFNCYFPLQSYGFQPTYGVGYQPYRVVVLSFELLHAPATVCGPKKSTNLVKNKCVNF

SEQ ID NO: 80 - protein, 223 aa, SARS-CoV-2
RVQPTESIVRFPNITNLCPFGEVFNATRFASVYAWNRKRISNCVADYSVLYNSASFSTFKCYGVSPTKLNDLCFTNVYADSFVIRGDEVRQIAPGQTGNIADYNYKLPDDFTGCVIAWNSNNLDSKVGGNYNYLYRLFRKSNLKPFERDISTEIYQAGSTPCNGVKGFNCYFPLQSYGFQPTYGVGYQPYRVVVLSFELLHAPATVCGPKKSTNLVKNKCVNF

SEQ ID NO: 81 - protein, 223 aa, SARS-CoV-2
RVQPTESIVRFPNITNLCPFGEVFNATRFASVYAWNRKRISNCVADYSVLYNSASFSTFKCYGVSPTKLNDLCFTNVYADSFVIRGDEVRQIAPGQTGTIADYNYKLPDDFTGCVIAWNSNNLDSKVGGNYNYLYRLFRKSNLKPFERDISTEIYQAGSTPCNGVKGFNCYFPLQSYGFQPTYGVGYQPYRVVVLSFELLHAPATVCGPKKSTNLVKNKCVNF

SEQ ID NO: 82 - protein, 223 aa, SARS-CoV-2
RVQPTESIVRFPNITNLCPFGEVFNATRFASVYAWNRKRISNCVADYSVLYNSASFSTFKCYGVSPTKLNDLCFTNVYADSFVIRGDEVRQIAPGQTGKIADYNYKLPDDFTGCVIAWNSNNLDSKVGGNYNYRYRLFRKSNLKPFERDISTEIYQAGSTPCNGVEGFNCYFPLQSYGFQPTNGVGYQPYRVVVLSFELLHAPATVCGPKKSTNLVKNKCVNF

SEQ ID NO: 83 - protein, 223 aa, SARS-CoV-2
RVQPTESIVRFPNITNLCPFGEVFNATRFASVYAWNRKRISNCVADYSVLYNSASFSTFKCYGVSPTKLNDLCFTNVYADSFVIRGDEVRQIAPGQTGKIADYNYKLPDDFTGCVIAWNSNNLDSKVGGNYNYRYRLFRKSNLKPFERDISTEIYQAGSTPCNGVQGFNCYFPLQSYGFQPTNGVGYQPYRVVVLSFELLHAPATVCGPKKSTNLVKNKCVNF

SEQ ID NO: 84 - protein, 223 aa, SARS-CoV-2
RVQPTESIVRFPNITNLCPFGEVFNATRFASVYAWNRKRISNCVADYSVLYNSASFSTFKCYGVSPTKLNDLCFTNVYADSFVIRGDEVRQIAPGQTGKIADYNYKLPDDFTGCVIAWNSNNLDSKVGGNYNYRYRLFRKSNLKPFERDISTEIYQAGSKPCNGVEGFNCYFPLQSYGFQPTNGVGYQPYRVVVLSFELLHAPATVCGPKKSTNLVKNKCVNF

SEQ ID NO: 85 - protein, 150 aa, Mus musculus
SRACPPCAPACKDNHCWGESPEDCQILTGTICTSGCARCKGRLPTDCCHEQCAAGCTGPKHSDCLACLHFNHSGICELHCPALVTYNTDTFESMHNPEGRYTFGASCVTTCPYNYLSTEVGSCTLVCPPNNQEVTAEDGTQRCEKCSKPC

SEQ ID NO: 86 - protein, 121 aa, Mus musculus
GCKKIFGSLAFLPESFDGDPSSGIAPLRPEQLQVFETLEEITGYLYISAWPDSLRDLSVFQNLRIIRGRILHDGAYSLTLQGLGIHSLGLRSLRELGSGLALIHRNAHLCFVHTVPWDQLF

SEQ ID NO: 87 - protein, 134 aa, Mus musculus
VCNSLCAHGHCWGPGPTQCVNCSHFLRGQECVEECRVWKGLPREYVSDKRCLPCHPECQPQNSSETCFGSEADQCAACAHYKDSSSCVARCPSGVKPDLSYMPIWKYPDEEGICQPCPINCTHSCVDLDERGCP

SEQ ID NO: 88 - protein, 150 aa, Homo sapiens
SRACHPCSPMCKGSRCWGESSEDCQSLTRTVCAGGCARCKGPLPTDCCHEQCAAGCTGPKHSDCLACLHFNHSGICELHCPALVTYNTDTFESMPNPEGRYTFGASCVTACPYNYLSTDVGSCTLVCPLHNQEVTAEDGTQRCEKCSKPC

SEQ ID NO: 89 - protein, 117 aa, Homo sapiens
GCKKIFGSLAFLPESFDGDPASNTAPLQPEQLQVFETLEEITGYLYISAWPDSLPDLSVFQNLQVIRGRILHNGAYSLTLQGLGISWLGLRSLRELGSGLALIHHNTHLCFVHTVPW

SEQ ID NO: 90 - protein, 133 aa, Homo sapiens
CHQLCARGHCWGPGPTQCVNCSQFLRGQECVEECRVLQGLPREYVNARHCLPCHPECQPQNGSVTCFGPEADQCVACAHYKDPPFCVARCPSGVKPDLSYMPIWKFPDEEGACQPCPINCTHSCVDLDDKGCP

SEQ ID NO: 91 - protein, 508 aa, Varicella zoster virus
SVLRYDDFHTDEDKLDTNSVYEPYYHSDHAESSWVNRGESSRKAYDHNSPYIWPRNDYDGFLENAHEHHGVYNQGRGIDSGERLMQPTQMSAQEDLGDDTGIHVIPTLNGDDRHKIVNVDQRQYGDVFKGDLNPKPQGQRLIEVSVEENHPFTLRAPIQRIYGVRYTETWSFLPSLTCTGDAAPAIQHICLKHTTCFQDVVVDVDCAENTKEDQLAEISYRFQGKKEADQPWIVVNTSTLFDELELDPPEIEPGVLKVLRTEKQYLGVYIWNMRGSDGTSTYATFLVTWKGDEKTRNPTPAVTPQPRGAEFHMWNYHSHVFSVGDTFSLAMHLQYKIHEAPFDLLLEWLYVPIDPTCQPMRLYSTCLYHPNAPQCLSHMNSGCTFTSPHLAQRVASTVYQNCEHADNYTAYCLGISHMEPSFGLILHDGGTTLKFVDTPESLSGLYVFVVYFNGHVEAVAYTVVSTVDHFVNAIEERGFPPTAGQPPATTKPKEITPVNPGTSPLLRY

SEQ ID NO: 92 - protein, 425 aa, Epstein-Barr virus
MEAALLVCQYTIQSLIHLTGEDPGFFNVEIPEFPFYPTCNVCTADVNVTINFDVGGKKHQLDLDFGQLTPHTKAVYQPRGAFGGSENATNLFLLELLGAGELALTMRSKKLPINVTTGEEQQVSLESVDVYFQDVFGTMWCHHAEMQNPVYLIPETVPYIKWDNCNSTNITAVVRAQGLDVTLPLSLPTSAQDSNFSVKTQMLGNEIDIECIMEDGEISQVLPGDNKFNITCSGYESHVPSGGILTSTSPVVTPIPGTGYAYSLRLTPRPVSRFLGNNSILYVFYSGNGPKASGGDYCIQSNIVFSDEIPASQDMPTNTTDITYVGDNATYSVPMVTSEDANSPNVTVTAFWAWPNNTETDFKCKWTLTSGTPSGCENISGAFASNRTFDITVSGLGTAPKTLIITRTATNATTTTHKVIFSKAP

SEQ ID NO: 93 - protein, 314 aa, Herpes simplex virus-2
KYALADPSLKMADPNRFRGKNLPVLDRLTDPPGVKRVYHIQPSLEDPFQPPSIPITVYYAVLERACRSVLLHAPSEAPQIVRGASDEARKHTYNLTIAWYRMGDNCAIPITVMEYTECPYNKSLGVCPIRTQPRWSYYDSFSAVSEDNLGFLMHAPAFETAGTYLRLVKINDWTEITQFILEHRARASCKYALPLRIPPAACLTSKAYQQGVTVDSIGMLPRFIPENQRTVALYSLKIAGWHGPKPPYTSTLLPPELSDTTNATQPELVPEDPEDSALLEDPAGTVSSQIPPNWHIPSIQDVAPHHAPAAPSNP